European Patent Application EP 4 180 811 A1, published May 17, 2023. Title: Methods of isolating a biological entity. Applicant: Cell.Copedia GmbH. The sequence listing filed with the application follows.

SEQUENCE LISTING (20 sequences)

SEQ ID NO: 1 - protein, 8 aa, synthetic construct
  REGION 1..8: note = streptavidin-binding peptide
  SITE 2: note = MISC_FEATURE - X is any amino acid
  SITE 7: note = MISC_FEATURE - X is Gly or Glu
  SITE 8: note = MISC_FEATURE - X is Gly, Lys or Arg
WXHPQFXX

SEQ ID NO: 2 - protein, 8 aa, synthetic construct
  REGION 1..8: note = streptavidin-binding peptide
WRHPQFGG

SEQ ID NO: 3 - protein, 8 aa, synthetic construct
  REGION 1..8: note = streptavidin-binding peptide
WSHPQFEK

SEQ ID NO: 4 - protein, 4 aa, synthetic construct
  REGION 1..4: note = streptavidin-binding peptide
HPQF

SEQ ID NO: 5 - protein, 8 aa, synthetic construct
  REGION 1..8: note = streptavidin-binding peptide
  SITE 1: note = MISC_FEATURE - X is Trp, Lys or Arg
  SITE 2: note = MISC_FEATURE - X is any amino acid
  SITE 7: note = MISC_FEATURE - X is Gly or Glu
  SITE 8: note = MISC_FEATURE - X is Gly, Lys or Arg
XXHPQFXX

SEQ ID NO: 6 - protein, 8 aa, synthetic construct
  REGION 1..8: note = streptavidin-binding peptide
  SITE 2: note = MISC_FEATURE - X is any amino acid
  SITE 7: note = MISC_FEATURE - X is Gly or Glu
  SITE 8: note = MISC_FEATURE - X is Gly, Lys or Arg
WXHPQFXX

SEQ ID NO: 7 - protein, 8 aa, synthetic construct
  REGION 1..8: note = streptavidin-binding peptide
WSHPQFEK

SEQ ID NO: 8 - protein, 28 aa, synthetic construct
  REGION 1..28: note = streptavidin-binding peptide
  REGION 9..20: note = MISC_FEATURE - X is any amino acid an up to 12 may be absent
WSHPQFEKXXXXXXXXXXXXWSHPQFEK

SEQ ID NO: 9 - protein, 8 aa, synthetic construct
  REGION 1..8: note = streptavidin-binding peptide
WSHPQFEK

SEQ ID NO: 10 - protein, 28 aa, synthetic construct
  REGION 1..28: note = streptavidin-binding peptide
WSHPQFEKGGGSGGGSGGGSWSHPQFEK

SEQ ID NO: 11 - protein, 24 aa, synthetic construct
  REGION 1..24: note = streptavidin-binding peptide
WSHPQFEKGGGSGGGSWSHPQFEK

SEQ ID NO: 12 - protein, 28 aa, synthetic construct
  REGION 1..28: note = streptavidin-binding peptide
WSHPQFEKGGGSGGGSGGSAWSHPQFEK

SEQ ID NO: 13 - protein, 4 aa, synthetic construct
  REGION 1..4: note = streptavidin mutein fragment
VTAR

SEQ ID NO: 14 - protein, 4 aa, synthetic construct
  REGION 1..4: note = streptavidin mutein fragment
IGAR

SEQ ID NO: 15 - protein, 9 aa, synthetic construct
  REGION 1..9: note = HA-tag
YPYDVPDYA

SEQ ID NO: 16 - protein, 11 aa, synthetic construct
  REGION 1..11: note = VSV-G-tag
YTDIEMNRLGK

SEQ ID NO: 17 - protein, 11 aa, synthetic construct
  REGION 1..11: note = HSV-tag
QPELAPEDPED

SEQ ID NO: 18 - protein, 10 aa, synthetic construct
  REGION 1..10: note = T7 epitope
ASMTGGQQMG

SEQ ID NO: 19 - protein, 10 aa, synthetic construct
  REGION 1..10: note = myc epitope of c-myc
EQKLISEEDL

SEQ ID NO: 20 - protein, 14 aa, synthetic construct
  REGION 1..14: note = V5 tag
GKPIPNPLLGLDST